European Patent Application EP 4 176 901 A1, published May 10, 2023. Title: STABLE COMPOSITIONS OF FOXY-5 HEXAPEPTIDE WITH HIGH SOLUBILITY. Applicant: WntResearch AB. The sequence listing filed with the application follows.

SEQUENCE LISTING (1 sequence)

SEQ ID NO: 1 - protein, 6 aa, Homo sapiens
MDGCEL